European Patent Application EP 4 520 748 A1, published March 12, 2025. Title: METHOD FOR PRODUCING SALT OF AMINO ACID OR SALT OF PEPTIDE COMPOUND OR SOLVATE THEREOF, COMPRISING PRECIPITATION STEP OF LITHIUM SALT. Applicant: CHUGAI SEIYAKU KABUSHIKI KAISHA. Application JP. The sequence listing filed with the application follows.

SEQUENCE LISTING (12 sequences)

SEQ ID NO: 1 - protein, 332 aa, Pseudomonas putida KT2440
MRVPFTELQSLLQAIFQRHGCSEAVARVLAHNCASAQRDGAHSHGVFRMPGYVSTLASGWVDGQATPQVSDVAAGYVRVDAAGGFAQPALAAARELLVAKARSAGIAVLAIHNSHHFAALWPDVEPFAEEGLVALSVVNSMTCVVPHGARKPLFGTNPIAFAAPCAEHDPIVFDMATSAMAHGDVQIAARAGQQLPEGMGVDADGQPTTDPKAILEGGALLPFGGHKGSALSMMVELLAAALTGGHFSWEFDWSGHPGAKTPWTGQLIIVIDPGKAEGQRFAQRSRELVEHMQAVGLTRMPGERRYREREVAEEEGVAVTEQELKGLKELLG

SEQ ID NO: 2 - protein, 332 aa, synthetic construct
  REGION 1..332: note = H44X
  VARIANT 44: note = A, R, N, D, C, Q, E, G, I, L, K, M, F, P, S, T, W, Y or V
MRVPFTELQSLLQAIFQRHGCSEAVARVLAHNCASAQRDGAHSXGVFRMPGYVSTLASGWVDGQATPQVSDVAAGYVRVDAAGGFAQPALAAARELLVAKARSAGIAVLAIHNSHHFAALWPDVEPFAEEGLVALSVVNSMTCVVPHGARKPLFGTNPIAFAAPCAEHDPIVFDMATSAMAHGDVQIAARAGQQLPEGMGVDADGQPTTDPKAILEGGALLPFGGHKGSALSMMVELLAAALTGGHFSWEFDWSGHPGAKTPWTGQLIIVIDPGKAEGQRFAQRSRELVEHMQAVGLTRMPGERRYREREVAEEEGVAVTEQELKGLKELLG

SEQ ID NO: 3 - protein, 332 aa, synthetic construct
  REGION 1..332: note = F117X
  VARIANT 117: note = A, R, N, D, C, Q, E, G, H, I, L, K, M, P, S, T, W, Y or V
MRVPFTELQSLLQAIFQRHGCSEAVARVLAHNCASAQRDGAHSHGVFRMPGYVSTLASGWVDGQATPQVSDVAAGYVRVDAAGGFAQPALAAARELLVAKARSAGIAVLAIHNSHHXAALWPDVEPFAEEGLVALSVVNSMTCVVPHGARKPLFGTNPIAFAAPCAEHDPIVFDMATSAMAHGDVQIAARAGQQLPEGMGVDADGQPTTDPKAILEGGALLPFGGHKGSALSMMVELLAAALTGGHFSWEFDWSGHPGAKTPWTGQLIIVIDPGKAEGQRFAQRSRELVEHMQAVGLTRMPGERRYREREVAEEEGVAVTEQELKGLKELLG

SEQ ID NO: 4 - protein, 332 aa, synthetic construct
  REGION 1..332: note = M141X
  VARIANT 141: note = A, R, N, D, C, Q, E, G, H, I, L, K, F, P, S, T, W, Y or V
MRVPFTELQSLLQAIFQRHGCSEAVARVLAHNCASAQRDGAHSHGVFRMPGYVSTLASGWVDGQATPQVSDVAAGYVRVDAAGGFAQPALAAARELLVAKARSAGIAVLAIHNSHHFAALWPDVEPFAEEGLVALSVVNSXTCVVPHGARKPLFGTNPIAFAAPCAEHDPIVFDMATSAMAHGDVQIAARAGQQLPEGMGVDADGQPTTDPKAILEGGALLPFGGHKGSALSMMVELLAAALTGGHFSWEFDWSGHPGAKTPWTGQLIIVIDPGKAEGQRFAQRSRELVEHMQAVGLTRMPGERRYREREVAEEEGVAVTEQELKGLKELLG

SEQ ID NO: 5 - protein, 332 aa, synthetic construct
  REGION 1..332: note = T156X
  VARIANT 156: note = A, R, N, D, C, Q, E, G, H, I, L, K, M, F, P, S, W, Y or V
MRVPFTELQSLLQAIFQRHGCSEAVARVLAHNCASAQRDGAHSHGVFRMPGYVSTLASGWVDGQATPQVSDVAAGYVRVDAAGGFAQPALAAARELLVAKARSAGIAVLAIHNSHHFAALWPDVEPFAEEGLVALSVVNSMTCVVPHGARKPLFGXNPIAFAAPCAEHDPIVFDMATSAMAHGDVQIAARAGQQLPEGMGVDADGQPTTDPKAILEGGALLPFGGHKGSALSMMVELLAAALTGGHFSWEFDWSGHPGAKTPWTGQLIIVIDPGKAEGQRFAQRSRELVEHMQAVGLTRMPGERRYREREVAEEEGVAVTEQELKGLKELLG

SEQ ID NO: 6 - protein, 332 aa, synthetic construct
  REGION 1..332: note = H182X
  VARIANT 182: note = A, R, N, D, C, Q, E, G, I, L, K, M, F, P, S, T, W, Y or V
MRVPFTELQSLLQAIFQRHGCSEAVARVLAHNCASAQRDGAHSHGVFRMPGYVSTLASGWVDGQATPQVSDVAAGYVRVDAAGGFAQPALAAARELLVAKARSAGIAVLAIHNSHHFAALWPDVEPFAEEGLVALSVVNSMTCVVPHGARKPLFGTNPIAFAAPCAEHDPIVFDMATSAMAXGDVQIAARAGQQLPEGMGVDADGQPTTDPKAILEGGALLPFGGHKGSALSMMVELLAAALTGGHFSWEFDWSGHPGAKTPWTGQLIIVIDPGKAEGQRFAQRSRELVEHMQAVGLTRMPGERRYREREVAEEEGVAVTEQELKGLKELLG

SEQ ID NO: 7 - protein, 332 aa, synthetic construct
  REGION 1..332: note = Q186X
  VARIANT 186: note = A, R, N, D, C, E, G, H, I, L, K, M, F, P, S, T, W, Y or V
MRVPFTELQSLLQAIFQRHGCSEAVARVLAHNCASAQRDGAHSHGVFRMPGYVSTLASGWVDGQATPQVSDVAAGYVRVDAAGGFAQPALAAARELLVAKARSAGIAVLAIHNSHHFAALWPDVEPFAEEGLVALSVVNSMTCVVPHGARKPLFGTNPIAFAAPCAEHDPIVFDMATSAMAHGDVXIAARAGQQLPEGMGVDADGQPTTDPKAILEGGALLPFGGHKGSALSMMVELLAAALTGGHFSWEFDWSGHPGAKTPWTGQLIIVIDPGKAEGQRFAQRSRELVEHMQAVGLTRMPGERRYREREVAEEEGVAVTEQELKGLKELLG

SEQ ID NO: 8 - protein, 332 aa, synthetic construct
  REGION 1..332: note = W253X
  VARIANT 253: note = A, R, N, D, C, Q, E, G, H, I, L, K, M, F, P, S, T, Y or V
MRVPFTELQSLLQAIFQRHGCSEAVARVLAHNCASAQRDGAHSHGVFRMPGYVSTLASGWVDGQATPQVSDVAAGYVRVDAAGGFAQPALAAARELLVAKARSAGIAVLAIHNSHHFAALWPDVEPFAEEGLVALSVVNSMTCVVPHGARKPLFGTNPIAFAAPCAEHDPIVFDMATSAMAHGDVQIAARAGQQLPEGMGVDADGQPTTDPKAILEGGALLPFGGHKGSALSMMVELLAAALTGGHFSWEFDXSGHPGAKTPWTGQLIIVIDPGKAEGQRFAQRSRELVEHMQAVGLTRMPGERRYREREVAEEEGVAVTEQELKGLKELLG

SEQ ID NO: 9 - protein, 332 aa, synthetic construct
  REGION 1..332: note = K260X
  VARIANT 260: note = A, R, N, D, C, Q, E, G, H, I, L, M, F, P, S, T, W, Y or V
MRVPFTELQSLLQAIFQRHGCSEAVARVLAHNCASAQRDGAHSHGVFRMPGYVSTLASGWVDGQATPQVSDVAAGYVRVDAAGGFAQPALAAARELLVAKARSAGIAVLAIHNSHHFAALWPDVEPFAEEGLVALSVVNSMTCVVPHGARKPLFGTNPIAFAAPCAEHDPIVFDMATSAMAHGDVQIAARAGQQLPEGMGVDADGQPTTDPKAILEGGALLPFGGHKGSALSMMVELLAAALTGGHFSWEFDWSGHPGAXTPWTGQLIIVIDPGKAEGQRFAQRSRELVEHMQAVGLTRMPGERRYREREVAEEEGVAVTEQELKGLKELLG

SEQ ID NO: 10 - protein, 375 aa, synthetic construct
  REGION 1..375: note = W253H-SBP tag-linker-His tag
MRVPFTELQSLLQAIFQRHGCSEAVARVLAHNCASAQRDGAHSHGVFRMPGYVSTLASGWVDGQATPQVSDVAAGYVRVDAAGGFAQPALAAARELLVAKARSAGIAVLAIHNSHHFAALWPDVEPFAEEGLVALSVVNSMTCVVPHGARKPLFGTNPIAFAAPCAEHDPIVFDMATSAMAHGDVQIAARAGQQLPEGMGVDADGQPTTDPKAILEGGALLPFGGHKGSALSMMVELLAAALTGGHFSWEFDHSGHPGAKTPWTGQLIIVIDPGKAEGQRFAQRSRELVEHMQAVGLTRMPGERRYREREVAEEEGVAVTEQELKGLKELLGGTDEKTTGWRGGHVVEGLAGELEQLRARLEHHPQGGSHHHHHH

SEQ ID NO: 11 - protein, 6 aa, synthetic construct
HHHHHH

SEQ ID NO: 12 - protein, 34 aa, synthetic construct
GTDEKTTGWRGGHVVEGLAGELEQLRARLEHHPQ